European Patent Specification EP 4 214 240 B1, published October 9, 2024. Title: Anti-CCR8 antibodies. Applicant: AbbVie Biotherapeutics Inc. Application US 63/226,118, filed July 27, 2021. The sequence listing filed with the application follows.

SEQUENCE LISTING (14 sequences)

SEQ ID NO: 1 - protein, 10 aa, synthetic construct
GFIFSNAVMY

SEQ ID NO: 2 - protein, 19 aa, synthetic construct
RIKTKFNNYATYYADAVKG

SEQ ID NO: 3 - protein, 9 aa, synthetic construct
GDRNKPFAY

SEQ ID NO: 4 - protein, 11 aa, synthetic construct
RASTSVITLLH

SEQ ID NO: 5 - protein, 7 aa, synthetic construct
GASNLES

SEQ ID NO: 6 - protein, 9 aa, synthetic construct
QQSWNDPYT

SEQ ID NO: 7 - protein, 120 aa, synthetic construct
EVQLVESGGGLVQPGGSLKLSCAASGFIFSNAVMYWVRQASGKGLEWVARIKTKFNNYATYYADAVKGRFTISRDDSKNMVYLQMNSLKTEDTAVYYCTAGDRNKPFAYWGQGTLVTVSS

SEQ ID NO: 8 - protein, 107 aa, synthetic construct
ETVVTQSPATLSLSPGERATLSCRASTSVITLLHWFQQKPGQAPRLLIHGASNLESRVPARFSGSGSGTDFTLTISSLEPEDFATYFCQQSWNDPYTFGQGTKLEIK

SEQ ID NO: 9 - protein, 450 aa, synthetic construct
EVQLVESGGGLVQPGGSLKLSCAASGFIFSNAVMYWVRQASGKGLEWVARIKTKFNNYATYYADAVKGRFTISRDDSKNMVYLQMNSLKTEDTAVYYCTAGDRNKPFAYWGQGTLVTVSSASTKGPSVFPLAPSSKSTSGGTAALGCLVKDYFPEPVTVSWNSGALTSGVHTFPAVLQSSGLYSLSSVVTVPSSSLGTQTYICNVNHKPSNTKVDKKVEPKSCDKTHTCPPCPAPELLGGPSVFLFPPKPKDTLMISRTPEVTCVVVDVSHEDPEVKFNWYVDGVEVHNAKTKPREEQYNSTYRVVSVLTVLHQDWLNGKEYKCKVSNKALPAPIEKTISKAKGQPREPQVYTLPPSREEMTKNQVSLTCLVKGFYPSDIAVEWESNGQPENNYKTTPPVLDSDGSFFLYSKLTVDKSRWQQGNVFSCSVMHEALHNHYTQKSLSLSPGK

SEQ ID NO: 10 - protein, 214 aa, synthetic construct
ETVVTQSPATLSLSPGERATLSCRASTSVITLLHWFQQKPGQAPRLLIHGASNLESRVPARFSGSGSGTDFTLTISSLEPEDFATYFCQQSWNDPYTFGQGTKLEIKRTVAAPSVFIFPPSDEQLKSGTASVVCLLNNFYPREAKVQWKVDNALQSGNSQESVTEQDSKDSTYSLSSTLTLSKADYEKHKVYACEVTHQGLSSPVTKSFNRGEC

SEQ ID NO: 11 - protein, 449 aa, synthetic construct
EVQLVESGGGLVQPGGSLKLSCAASGFIFSNAVMYWVRQASGKGLEWVARIKTKFNNYATYYADAVKGRFTISRDDSKNMVYLQMNSLKTEDTAVYYCTAGDRNKPFAYWGQGTLVTVSSASTKGPSVFPLAPSSKSTSGGTAALGCLVKDYFPEPVTVSWNSGALTSGVHTFPAVLQSSGLYSLSSVVTVPSSSLGTQTYICNVNHKPSNTKVDKKVEPKSCDKTHTCPPCPAPELLGGPSVFLFPPKPKDTLMISRTPEVTCVVVDVSHEDPEVKFNWYVDGVEVHNAKTKPREEQYNSTYRVVSVLTVLHQDWLNGKEYKCKVSNKALPAPIEKTISKAKGQPREPQVYTLPPSREEMTKNQVSLTCLVKGFYPSDIAVEWESNGQPENNYKTTPPVLDSDGSFFLYSKLTVDKSRWQQGNVFSCSVMHEALHNHYTQKSLSLSPG

SEQ ID NO: 12 - DNA, 1410 bp, synthetic construct
  source 1..1410: mol_type = other DNA
atggaattcggcctgagctggctgttcctggtggccatcctgaagggcgtgcagtgcgaagtccagctggttgaatctggcggaggactggttcagcctggcggatctctgaagctgtcttgtgccgccagcggcttcatcttcagcaacgccgtgatgtactgggtccgacaggcctctggcaaaggcctggaatgggtcgccagaatcaagaccaagttcaacaactacgccacctactacgccgacgccgtgaagggcagattcaccatcagcagggacgacagcaagaacatggtgtacctgcagatgaacagcctgaaaaccgaggacaccgccgtgtactactgcacagccggcgacagaaacaagccctttgcctattggggccagggcaccctggttaccgttagctctgcctccaccaagggcccatcggtcttccccctggcaccctcctccaagagcacctctgggggcacagcggccctgggctgcctggtcaaggactacttccccgaaccggtgacggtgtcgtggaactcaggcgccctgaccagcggcgtgcacaccttcccggctgtcctacagtcctcaggactctactccctcagcagcgtggtgaccgtgccctccagcagcttgggcacccagacctacatctgcaacgtgaatcacaagcccagcaacaccaaggtggacaagaaagttgagcccaaatcttgtgacaaaactcacacatgcccaccgtgcccagcacctgaactcctggggggaccgtcagtcttcctcttccccccaaaacccaaggacaccctcatgatctcccggacccctgaggtcacatgcgtggtggtggacgtgagccacgaagaccctgaggtcaagttcaactggtacgtggacggcgtggaggtgcataatgccaagacaaagccgcgggaggagcagtacaacagcacgtaccgtgtggtcagcgtcctcaccgtcctgcaccaggactggctgaatggcaaggagtacaagtgcaaggtctccaacaaagccctcccagcccccatcgagaaaaccatctccaaagccaaagggcagccccgagaaccacaggtgtacaccctgcccccatcccgggaggagatgaccaagaaccaggtcagcctgacctgcctggtcaaaggcttctatcccagcgacatcgccgtggagtgggagagcaatgggcagccggagaacaactacaagaccacgcctcccgtgctggactccgacggctccttcttcctctacagcaagctcaccgtggacaagagcaggtggcagcaggggaacgtcttctcatgctccgtgatgcatgaggctctgcacaaccactacacgcagaagagcctctccctgtctccgggcaaatga

SEQ ID NO: 13 - DNA, 711 bp, synthetic construct
  source 1..711: mol_type = other DNA
atggacatgcgggtgcccgcccagctgctgggacttctgctgctgtggttccccggcagcagatgcgagacagtggtcacacagtctcccgccacactgtcactgtctccaggcgaaagagccacactgagctgtagagccagcaccagcgtgatcacactgctgcactggttccagcagaagcctggacaggctcccagactgctgattcacggcgccagcaacctggaaagcagagtgcctgccagattttccggcagcggctctggcaccgatttcaccctgaccataagcagcctggaacctgaggacttcgccacctacttttgccagcagagctggaacgacccctacacctttggccagggcaccaagctggaaatcaagcgaactgtggctgcaccatctgtcttcatcttcccgccatctgatgagcagttgaaatctggaactgcctctgttgtgtgcctgctgaataacttctatcccagagaggccaaagtacagtggaaggtggataacgccctccaatcgggtaactcccaggagagtgtcacagagcaggacagcaaggacagcacctacagcctcagcagcaccctgacgctgagcaaagcagactacgagaaacacaaagtctacgcctgcgaagtcacccatcagggcctgagctcgcccgtcacaaagagcttcaacaggggagagtgttag

SEQ ID NO: 14 - protein, 12 aa, synthetic construct
CTAGDRNKPFAY